European Patent Specification EP 3 515 504 B1, published July 12, 2023. Title: CANINE ADENOVIRUS VECTORS. Applicant: Boehringer Ingelheim Vetmedica GmbH. The sequence listing filed with the application follows.

SEQUENCE LISTING (47 sequences)

SEQ ID NO: 1 - DNA, 1010 bp, Canine adenovirus type 2
ctcccaaataggtataaaaagcccagtgctggctggcacgggcattcagcttagcgaagacatccccagcgcctcctggatcaggcccgacggcatattccagctaggaggggggtctcgctcgtccttcagcccaacgcaagcattcctcaccctgcaacaggcatcctcgacgccgcgcgcaggaggcgtgggcacctaccagtttgtgcgcgaatttgtgccagaggtataccttaaccctttttcaggaccaccggacacctttcctgatcagttcattcctaactacgacattgtaaccaactctgtcgatggctatgactgaggagagcatggaccaggtggaggtgaactgcctgtgtgctcagcatgcccaaacctgcacgcgccctcgctgctttgcaaaggagggtttatgtgctaactggttttacaacccagcacttgcctttgaagggtttgatattccagactcttaccaagagggacacggtgtgattcccagagtgcgtcctcaacatcacccgcgacggaactttcctgcttattggggatagcaaaaagaccccctatgtcatcctgctgcccttttttgcaaaccccaaagaagacactccaattttaatggcccttagccattccatgcccgtcgccatacctgacactgcaatgcctatatatatttccatcatgttttttattgtggccatgctagccaccctcagccttctaatgggactaaacaacaaaaatcaggcccatgtagcttgtcaaataaacttacctaatttttgctaagacgtctgggtcctgcgtttctatgtccaccaaagtcccctcttcccagctttggtacttccacttgtgcgcgcgagccagcttgcggatgtgcttgaaagataatgtggtctctcccaacagcttcccgttcaccagcaccagggccatgaagcggacacgaagagctctacctgcaaattatgaccctgtatatccatacgacgccc

SEQ ID NO: 2 - DNA, 1011 bp, Canine adenovirus type 2
ctcccaaataggtataaaaagcccagtgctggctggcacgggcattcagcttagcgaagacatccccagcgcctcctggatcaggcccgacggcatattccagctaggaggggggtctcgctcgtccttcagcccaacgcaagcattcctcaccctgcaacaggcatcctcgacgccgcgcgcaggaggcgtgggcacctaccagtttgtgcgcgaatttgtgccagaggtataccttaaccctttttcaggaccaccggacacctttcctgatcagttcattcctaactacgacattgtaaccaactctgtcgatggctatgactgaggagagcatggaccaggtggaggtgaactgcctgtgtgctcagcatgcccaaacctgcacgcgccctcgctgctttgcaaaggagggtttatgtgctaactggttttacaacccagcacttgcctttgaagggtttgatattccagactcttaccaagagggacacggtgtgacaccctcagccttctaatgggactaaacaacaaaaatcaggcccatgtagcttgtcaaataaacttacctaatttttgctaagacgtctgggtcctgcgtttctatgtccaccaaagtcccctcttcccagctttggtacttccacttgtgcgcgcgagccagcttgcggatgtgcttgaaagataatgtggtctctcccaacagcttcccgttcaccagcaccagggccatgaagcggacacgaagagctctacctgcaaattatgaccctgtatatccatacgacgcccccgggtcttccacacaaccccctttttttaataacaagcaaggtctcactgagtcacccccaggaaccctggctgtcaatgtttcccctccactaaccttttctacgttaggtgccattaaactttccacaggtcccggactcaccctcaacgagggcaagttacaagccagcttagggcccggcctcatcacaaataccgagggccaaatcactgttg

SEQ ID NO: 3 - DNA, 545 bp, Artificial Sequence
  NUCLEOTIDE SEQUENCE FROM HUMAN CMV PROMOTER
ttattaatagtaatcaattacggggtcattagttcatagcccatatatggagttccgcgttacataacttacggtaaatggcccgcctggctgaccgcccaacgacccccgcccattgacgtcaataatgacgtatgttcccatagtaacgccaatagggactttccattgacgtcaatgggtggagtatttacggtaaactgcccacttggcagtacatcaagtgtatcatatgccaagtacgccccctattgacgtcaatgacggtaaatggcccgcctggcattatgcccagtacatgaccttatgggactttcctacttggcagtacatctacgtattagtcatcgctattaccatggtgatgcggttttggcagtacatcaatgggcgtggatagcggtttgactcacggggatttccaagtctccaccccattgacgtcaatgggagtttgttttggcaccaaaatcaacgggactttccaaaatgtcgtaacaactccgccccattgacgcaaatgggcggtaggcgtgtacggtggc

SEQ ID NO: 4 - DNA, 1110 bp, Artificial Sequence
  NUCLEOTIDE SEQUENCE FROM HUMAN CMV PROMOTER AND AD5 LEADER
ttattaatagtaatcaattacggggtcattagttcatagcccatatatggagttccgcgttacataacttacggtaaatggcccgcctggctgaccgcccaacgacccccgcccattgacgtcaataatgacgtatgttcccatagtaacgccaatagggactttccattgacgtcaatgggtggagtatttacggtaaactgcccacttggcagtacatcaagtgtatcatatgccaagtacgccccctattgacgtcaatgacggtaaatggcccgcctggcattatgcccagtacatgaccttatgggactttcctacttggcagtacatctacgtattagtcatcgctattaccatggtgatgcggttttggcagtacaccaatgggcgtggatagcggtttgactcacggggatttccaagtctccaccccattgacgtcaatgggagtttgttttggcaccaaaatcaacgggactttccaaaatgtcgtaataaccccgccccgttgacgcaaatgggcggtaggcgtgtacggtgggaggtctatataagcagagctcgtttagtgaaccgtcagatcctcactctcttccgcatcgctgtctgcgagggccagctgttgggctcgcggttgaggacaaactcttcgcggtctttccagtactcttggatcggaaacccgtcggcctccgaacggtactccgccaccgagggacctgagccagtccgcatcgaccggatcggaaaacctctcgagaaaggcgtctaaccagtcacagtcgcaaggtaggctgagcaccgtggcgggcggcagcgggtggcggtcggggttgtttctggcggaggtgctgctgatgatgtaattaaagtaggcggtcttgagccggcggatggtcgaggtgaggtgtggcaggcttgagatccagctgttggggtgagtactccctctcaaaagcgggcatgacttctgcgctaagattgtcagtttccaaaaacgaggaggatttgatattcacctggcccgatctggccatacacttgagtgacaatgacatccactttgcctttctctccacaggtgtccactcccaggtccaagtataa

SEQ ID NO: 5 - DNA, 25 bp, Artificial Sequence
  PRIMER
ttattaatagtaatcaattacgggg

SEQ ID NO: 6 - DNA, 23 bp, Artificial Sequence
  PRIMER
gccaccgtacacgcctaccgccc

SEQ ID NO: 7 - DNA, 1570 bp, Artificial Sequence
  NUCLEOTIDE SEQUENCE OF TRANSFER PLASMID CMVie EGFP  EXPRESSION CASSETTE
ttattaatagtaatcaattacggggtcattagttcatagcccatatatggagttccgcgttacataacttacggtaaatggcccgcctggctgaccgcccaacgacccccgcccattgacgtcaataatgacgtatgttcccatagtaacgccaatagggactttccattgacgtcaatgggtggagtatttacggtaaactgcccacttggcagtacatcaagtgtatcatatgccaagtacgccccctattgacgtcaatgacggtaaatggcccgcctggcattatgcccagtacatgaccttatgggactttcctacttggcagtacatctacgtattagtcatcgctattaccatggtgatgcggttttggcagtacatcaatgggcgtggatagcggtttgactcacggggatttccaagtctccaccccattgacgtcaatgggagtttgttttggcaccaaaatcaacgggactttccaaaatgtcgtaacaactccgccccattgacgcaaatgggcggtaggcgtgtacggtggcggatccgccgccaccatgggccgccaccatggtgagcaagggcgaggagctgttcaccggggtggtgcccatcctggtcgagctggacggcgacgtaaacggccacaagttcagcgtgtccggcgagggcgagggcgatgccacctacggcaagctgaccctgaagttcatctgcaccaccggcaagctgcccgtgccctggcccaccctcgtgaccaccctgacctacggcgtgcagtgcttcagccgctaccccgaccacatgaagcagcacgacttcttcaagtccgccatgcccgaaggctacgtccaggagcgcaccatcttcttcaaggacgacggcaactacaagacccgcgccgaggtgaagttcgagggcgacaccctggtgaaccgcatcgagctgaagggcatcgacttcaaggaggacggcaacatcctggggcacaagctggagtacaactacaacagccacaacgtctatatcatggccgacaagcagaagaacggcatcaaggtgaacttcaagatccgccacaacatcgaggacggcagcgtgcagctcgccgaccactaccagcagaacacccccatcggcgacggccccgtgctgctgcccgacaaccactacctgagcacccagtccgccctgagcaaagaccccaacgagaagcgcgatcacatggtcctgctggagttcgtgaccgccgccgggatcactctcggcatggacgagctgtacaagtaagtcgactatttcgagtacctctagggccgcttcgagcagacatgataagatacattgatgagtttggacaaaccacaactagaatgcagtgaaaaaaatgctttatttgtgaaatttgtgatgctattgctttatttgtaaccattataagctgcaataaacaagttaacaacaacaattgcattcattttatgtttcaggttcagggggagatgtgggaggttttttaaagcaagtaaaacctctacaaatgtggtaaaatcgaatctagatcctc

SEQ ID NO: 8 - DNA, 19 bp, Artificial Sequence
  PRIMER
gggcgaggagctgttcacc

SEQ ID NO: 9 - DNA, 21 bp, Artificial Sequence
  PRIMER
ccggcggcggtcacgaactcc

SEQ ID NO: 10 - DNA, 3636 bp, Artificial Sequence
  NUCLEOTIDE SEQUENCE OF TRANSFER PLASMID CMVie CPV VP2 (n) EXPRESSION CASSETTE
ccacgtggtttaaacctcccaaataggtataaaaagcccagtgctggctggcacgggcattcagcttagcgaagacatccccagcgcctcctggatcaggcccgacggcatattccagctaggaggggggtctcgctcgtccttcagcccaacgcaagcattcctcaccctgcaacaggcatcctcgacgccgcgcgcaggaggcgtgggcacctaccagtttgtgcgcgaatttgtgccagaggtataccttaaccctttttcaggaccaccggacacctttcctgatcagttcattcctaactacgacattgtaaccaactctgtcgatggctatgactgaggagagcatggaccaggtggaggtgaactgcctgtgtgctcagcatgcccaaacctgcacgcgccctcgctgctttgcaaaggagggtttatgtgctaactggttttacaacccagcacttgcctttgaagggtttgatattccagactcttaccaagagggacacggtgtggtacctagttattaatagtaatcaattacggggtcattagttcatagcccatatatggagttccgcgttacataacttacggtaaatggcccgcctggctgaccgcccaacgacccccgcccattgacgtcaataatgacgtatgttcccatagtaacgccaatagggactttccattgacgtcaatgggtggagtatttacggtaaactgcccacttggcagtacatcaagtgtatcatatgccaagtacgccccctattgacgtcaatgacggtaaatggcccgcctggcattatgcccagtacatgaccttatgggactttcctacttggcagtacatctacgtattagtcatcgctattaccatggtgatgcggttttggcagtacatcaatgggcgtggatagcggtttgactcacggggatttccaagtctccaccccattgacgtcaatgggagtttgttttggcaccaaaatcaacgggactttccaaaatgtcgtaacaactccgccccattgacgcaaatgggcggtaggcgtgtacggtggcggatccgccgccaccatgagtgatggagcagttcaaccagacggtggtcaacctgctgtcagaaatgaaagagctacaggatctgggaacgggtctggaggcgggggtggtggtggttctgggggtgtggggatttctacgggtactttcaataatcagacggaatttaaatttttggaaaacggatgggtggaaatcacagcaaactcaagcagacttgtacatttaaatatgccagaaagtgaaaattatagaagagtggttgtaaataatttggataaaactgcagttaacggaaacatggctttagatgatactcatgcacaaattgtaacaccttggtcattggttgatgcaaatgcttggggagtttggtttaatccaggagattggcaactaattgttaatactatgagtgagttgcatttagttagttttgaacaagaaatttttaatgttgttttaaagactgtttcagaatctgctactcagccaccaactaaagtttataataatgatttaactgcatcattgatggttgcattagatagtaataatactatgccatttactccagcagctatgagatctgagacattgggtttttatccatggaaaccaaccataccaactccatggagatattattttcaatgggatagaacattaataccatctcatactggaactagtggcacaccaacaaatatataccatggtacagatccagatgatgttcaattttatactattgaaaattctgtgccagtacacttactaagaacaggtgatgaatttgctacaggaacatttttttttgattgtaaaccatgtagactaacacatacatggcaaacaaatagagcattgggcttaccaccatttctaaattctttgcctcaagctgaaggaggtactaactttggttatataggagttcaacaagataaaagacgtggtgtaactcaaatgggaaaaacaaactatattactgaagctactattatgagaccagctgaggttggttatagtgcaccatattattcttttgaggcgtctacacaagggccatttaaaacacctattgcagcaggacgggggggagcgcaaacagatgaaaatcaaggagcagatggtaatccaagatatgcatttggtagacaacatggtcaaaaaactaccacaacaggagaaacacctgagagatttacatatatagcacatcaagatacaggaagatatccagaaggagattggattcaaaatattaactttaaccttcctgtaacagatgataatgtattgctaccaacagatccaattggaggtaaaacaggaattaactatactaatatatttaatacttatggtcctttaactgcattaaataatgtaccaccagtttatccaaatggtcaaatttgggataaagaatttgatactgacttaaaaccaagacttcatgtaaatgcaccatttgtttgtcaaaataattgtcctggtcaattatttgtaaaagttgcgcctaatttaacaaatgaatatgatcctgatgcatctgctaatatgtcaagaattgtaacttactcagatttttggtggaaaggtaaattagtatttaaagctaaactaagagcctctcatacttggaatccaattcaacaaatgagtattaatgtagataaccaatttaactatgtaccaagtaatattggaggtatggaaattgtatttgaaagatctcaactagcacctagaaaattatattaagtcgactatttcgagtacctctagggccgcttcgagcagacatgataagatacattgatgagtttggacaaaccacaactagaatgcagtgaaaaaaatgctttatttgtgaaatttgtgatgctattgctttatttgtaaccattataagctgcaataaacaagttaacaacaacaattgcattcattttatgtttcaggttcagggggagatgtgggaggttttttaaagcaagtaaaacctctacaaatgtggtaaaatcgaatctagatcctccttaagacaccctcagccttctaatgggactaaacaacaaaaatcaggcccatgtagcttgtcaaataaacttacctaatttttgctaagacgtctgggtcctgcgtttctatgtccaccaaagtcccctcttcccagctttggtacttccacttgtgcgcgcgagccagcttgcggatgtgcttgaaagataatgtggtctctcccaacagcttcccgttcaccagcaccagggccatgaagcggacacgaagagctctacctgcaaattatgaccctgtatatccatacgacgcccccgggtcttccacacaaccccctttttttaataacaagcaaggtctcactgagtcacccccaggaaccctggctgtcaatgtttcccctccactaaccttttctacgttaggtgccattaaactttccacaggtcccggactcaccctcaacgagggcaagttacaagccagcttagggcccggcctcatcacaaataccgagggccaaatcactgttggttt

SEQ ID NO: 11 - DNA, 28 bp, Artificial Sequence
  PRIMER
tgatcagttcattcctaactacgacatt

SEQ ID NO: 12 - DNA, 22 bp, Artificial Sequence
  PRIMER
ttgctatctaatgcaaccatca

SEQ ID NO: 13 - DNA, 20 bp, Artificial Sequence
  PRIMER
aatgcaccatttgtttgtca

SEQ ID NO: 14 - DNA, 21 bp, Artificial Sequence
  PRIMER
gggaagctgttgggagagacc

SEQ ID NO: 15 - DNA, 19 bp, Artificial Sequence
  PRIMER
aatgcttggggagtttggt

SEQ ID NO: 16 - DNA, 20 bp, Artificial Sequence
  PRIMER
ttgtgtagacgcctcaaaag

SEQ ID NO: 17 - DNA, 19 bp, Artificial Sequence
  PRIMER
aatgcttggggagtttggt

SEQ ID NO: 18 - DNA, 22 bp, Artificial Sequence
  PRIMER
tgcatcaggatcatattcattt

SEQ ID NO: 19 - DNA, 23 bp, Artificial Sequence
  PRIMER
aactcaaatgggaaatacaaact

SEQ ID NO: 20 - DNA, 22 bp, Artificial Sequence
  PRIMER
tgcatcaggatcatattcattt

SEQ ID NO: 21 - DNA, 28 bp, Artificial Sequence
  PRIMER
tgatcagttcattcctaactacgacatt

SEQ ID NO: 22 - DNA, 21 bp, Artificial Sequence
  PRIMER
gggaagctgttgggagagacc

SEQ ID NO: 23 - DNA, 2563 bp, Artificial Sequence
  NUCLEOTIDE SEQUENCE OF TRANSFER PLASMID CMVie CPV VP2 (co) EXPRESSION CASSETTE
ttattaatagtaatcaattacggggtcattagttcatagcccatatatggagttccgcgttacataacttacggtaaatggcccgcctggctgaccgcccaacgacccccgcccattgacgtcaataatgacgtatgttcccatagtaacgccaatagggactttccattgacgtcaatgggtggagtatttacggtaaactgcccacttggcagtacatcaagtgtatcatatgccaagtacgccccctattgacgtcaatgacggtaaatggcccgcctggcattatgcccagtacatgaccttatgggactttcctacttggcagtacatctacgtattagtcatcgctattaccatggtgatgcggttttggcagtacatcaatgggcgtggatagcggtttgactcacggggatttccaagtctccaccccattgacgtcaatgggagtttgttttggcaccaaaatcaacgggactttccaaaatgtcgtaacaactccgccccattgacgcaaatgggcggtaggcgtgtacggtggcggatccgccgccaccatgtctgatggcgccgtgcagcctgatggcggacagcctgctgtgcggaatgagagagccaccggcagcggcaatggatctggcggaggcggcggagggggaagtggcggagtgggaattagcaccggcaccttcaacaaccagaccgagttcaagttcctggaaaacggctgggtggaaatcaccgccaacagcagcagactggtgcacctgaacatgcccgagagcgagaactaccggcgggtggtcgtgaacaacctggacaagaccgccgtgaacggcaacatggccctggacgatacccacgcccagatcgtgacaccctggtccctggtggatgccaatgcctggggcgtgtggttcaaccccggcgactggcagctgatcgtgaacaccatgagcgagctgcacctggtgtccttcgagcaggaaatcttcaacgtggtgctgaaaaccgtgtccgagagcgccacacagccccccaccaaggtgtacaacaacgacctgaccgcctccctgatggtggctctggacagcaacaacaccatgcccttcacccctgccgccatgcggagcgagacactgggcttctacccctggaagcccaccatccctaccccctggcggtactacttccagtgggacagaaccctgatccccagccacacaggcaccagcggcacccctaccaacatctaccacggcaccgaccccgacgacgtgcagttctacaccatcgagaacagcgtgcccgtgcatctgctgagaaccggcgacgagttcgccacaggcacattctttttcgactgcaaaccctgccggctgacccacacctggcagaccaatagagccctgggcctgcccccattcctgaacagtctgcctcaggccgagggcggcaccaactttggctatatcggcgtgcagcaggacaagcggagaggcgtgacacagatgggcaagaccaactacatcaccgaggccacaatcatgcggcctgccgaagtgggctacagcgccccctactacagcttcgaggccagcacccagggccccttcaagacacctattgccgccggaagaggcggagcccagaccgatgagaatcagggcgccgacggcaaccccagatacgcctttggcagacagcacggccagaaaaccaccaccaccggcgagacacccgagcggttcacctatatcgcccaccaggacaccggcagataccccgagggcgactggattcagaacatcaacttcaacctgcccgtgaccgacgacaacgtgctgctgcccacagatcccatcggcggcaagaccggcatcaactacaccaatatcttcaacacctacggccctctgaccgccctgaacaacgtgccccccgtgtaccccaacggacagatctgggacaaagagttcgacaccgacctgaagccccggctgcatgtgaacgcccctttcgtgtgccagaacaactgccctggccagctgtttgtgaaggtggcccccaacctgaccaacgagtacgaccctgacgccagcgccaacatgagccggatcgtgacctacagcgacttctggtggaagggcaagctggtgttcaaggccaagctgcgggcctctcacacctggaaccccatccagcagatgagcatcaacgtggacaaccagttcaactacgtgcccagcaacatcggcggaatggaaatcgtgttcgagcggtcccagctggcccccagaaagctgtactaatctagagggccctattctatagtgtcacctaaatgctagagctcgctgatcagcctcgactgtgccttctagttgccagccatctgttgtttgcccctcccccgtgccttccttgaccctggaaggtgccactcccactgtcctttcctaataaaatgaggaaattgcatcgcattgtctgagtaggtgtcattctattctggggggtggggtggggcaggacagcaagggggaggattgggaagaca

SEQ ID NO: 24 - protein, 584 aa, canine parvovirus
MSDGAVQPDGGQPAVRNERATGSGNGSGGGGGGGSGGVGISTGTFNNQTEFKFLENGWVEITANSSRLVHLNMPESENYRRVVVNNLDKTAVNGNMALDDTHAQIVTPWSLVDANAWGVWFNPGDWQLIVNTMSELHLVSFEQEIFNVVLKTVSESATQPPTKVYNNDLTASLMVALDSNNTMPFTPAAMRSETLGFYPWKPTIPTPWRYYFQWDRTLIPSHTGTSGTPTNIYHGTDPDDVQFYTIENSVPVHLLRTGDEFATGTFFFDCKPCRLTHTWQTNRALGLPPFLNSLPQAEGGTNFGYIGVQQDKRRGVTQMGKTNYITEATIMRPAEVGYSAPYYSFEASTQGPFKTPIAAGRGGAQTDENQGADGNPRYAFGRQHGQKTTTTGETPERFTYIAHQDTGRYPEGDWIQNINFNLPVTDDNVLLPTDPIGGKTGINYTNIFNTYGPLTALNNVPPVYPNGQIWDKEFDTDLKPRLHVNAPFVCQNNCPGQLFVKVAPNLTNEYDPDASANMSRIVTYSDFWWKGKLVFKAKLRASHTWNPIQQMSINVDNQFNYVPSNIGGMEIVFERSQLAPRKLY

SEQ ID NO: 25 - DNA, 2418 bp, Artificial Sequence
  NUCLEOTIDE SEQUENCE OF TRANSFER PLASMID CMVie RabGP (n) EXPRESSION CASSETTE
ttattaatagtaatcaattacggggtcattagttcatagcccatatatggagttccgcgttacataacttacggtaaatggcccgcctggctgaccgcccaacgacccccgcccattgacgtcaataatgacgtatgttcccatagtaacgccaatagggactttccattgacgtcaatgggtggagtatttacggtaaactgcccacttggcagtacatcaagtgtatcatatgccaagtacgccccctattgacgtcaatgacggtaaatggcccgcctggcattatgcccagtacatgaccttatgggactttcctacttggcagtacatctacgtattagtcatcgctattaccatggtgatgcggttttggcagtacatcaatgggcgtggatagcggtttgactcacggggatttccaagtctccaccccattgacgtcaatgggagtttgttttggcaccaaaatcaacgggactttccaaaatgtcgtaacaactccgccccattgacgcaaatgggcggtaggcgtgtacggtggcggatccgccgccaccatggtaccggttcctcaggctctcctgtttgtaccccttctggtttttccattgtgttttgggaaattccctatttacacgataccagacaagcttggtccctggagcccgattgacatacatcacctcagctgcccaaacaatttggtagtggaggacgaaggatgcaccaacctgtcagggttctcctacatggaacttaaagttggatacatctcagccataaaaatgaacgggttcacttgcacaggcgttgtgacggaggctgaaacctacactaacttcgttggttatgtcacaaccacgttcaaaagaaagcatttccgcccaacaccagatgcatgtagagccgcgtacaactggaagatggccggtgaccccagatatgaagagtctctacacaatccgtaccctgactaccactggcttcgaactgtaaaaaccaccaaggagtctctcgttatcatatctccaagtgtggcagatttggacccatatgacagatcccttcactcgagggtcttccctggcgggaagtgctcaggagtagcggtgtcttctacctactgctccactaaccacgattacaccatttggatgcccgagaatccgagactagggatgtcttgtgacatttttaccaatagtagagggaagagagcatccaaagggagtgagacttgcggctttgtagatgaaagaggcctatataagtctttaaaaggagcatgcaaactcaagttatgtggagttctcggacttagacttatggatggaacatgggtctcgatgcaaacatcaaatgaaaccaaatggtgccctcccggtcagttgatcaatttgcacgactttcgctcagacgaaattgagcaccttgttgtagaggagttggtcaagaagagagaggagtgtctggatgcactagagtccatcatgaccaccaagtcagtaagtttcagacgtctcagtcatttaagaaaacttgtccctgggtttggaaaagcatataccatattcaacaagaccttgatggaagccgatgctcactacaagtcagtcagaacttggaatgagatcatcccttcaaaagggtgtttaagagttggggggaggtgtcatcctcatgtaaacggggtatttttcaatggtataatattaggacctgacggcaatgtcttaatcccagagatgcaatcatccctcctccagcaacatatggagttgttggtatcctcggttatcccccttatgcaccccctggcagacccgtctaccgttttcaagaacggtgacgaggctgaggattttgttgaagttcaccttcccgatgtgcacgaacggatctcaggagttgacttgggtctcccgaactgggggaagtatgtattactgagtgcaggggccctgactgccttgatgttgataattttcctgatgacatgctggagaagagtcaatcgatcggaacctacacaacacaatctcagagggacagggagggaggtgtcagtcactccccaaagcgggaagatcatatcttcatgggaatcatacaagagcgggggtgagaccggactgtgagtcgactatttcgagtacctctagggccgcttcgagcagacatgataagatacattgatgagtttggacaaaccacaactagaatgcagtgaaaaaaatgctttatttgtgaaatttgtgatgctattgctttatttgtaaccattataagctgcaataaacaagttaacaacaacaattgcattcattttatgtttcaggttcagggggagatgtgggaggttttttaaagcaagtaaaacctctacaaatgtggtaaaatcgaatctagatcctc

SEQ ID NO: 26 - protein, 526 aa, Rabies virus
MVPVPQALLFVPLLVFPLCFGKFPIYTIPDKLGPWSPIDIHHLSCPNNLVVEDEGCTNLSGFSYMELKVGYISAIKMNGFTCTGVVTEAETYTNFVGYVTTTFKRKHFRPTPDACRAAYNWKMAGDPRYEESLHNPYPDYHWLRTVKTTKESLVIISPSVADLDPYDRSLHSRVFPGGKCSGVAVSSTYCSTNHDYTIWMPENPRLGMSCDIFTNSRGKRASKGSETCGFVDERGLYKSLKGACKLKLCGVLGLRLMDGTWVSMQTSNETKWCPPGQLINLHDFRSDEIEHLVVEELVKKREECLDALESIMTTKSVSFRRLSHLRKLVPGFGKAYTIFNKTLMEADAHYKSVRTWNEIIPSKGCLRVGGRCHPHVNGVFFNGIILGPDGNVLIPEMQSSLLQQHMELLVSSVIPLMHPLADPSTVFKNGDEAEDFVEVHLPDVHERISGVDLGLPNWGKYVLLSAGALTALMLIIFLMTCWRRVNRSEPTQHNLRGTGREVSVTPQSGKIISSWESYKSGGETGL

SEQ ID NO: 27 - DNA, 3546 bp, Artificial Sequence
  NUCLEOTIDE SEQUENCE OF TRANSFER PLASMID CMVie BRSV F (co) EXPRESSION CASSETTE
tcagcttagcgaagacatccccagcgcctcctggatcaggcccgacggcatattccagctaggaggggggtctcgctcgtccttcagcccaacgcaagcattcctcaccctgcaacaggcatcctcgacgccgcgcgcaggaggcgtgggcacctaccagtttgtgcgcgaatttgtgccagaggtataccttaaccctttttcaggaccaccggacacctttcctgatcagttcattcctaactacgacattgtaaccaactctgtcgatggctatgactgaggagagcatggaccaggtggaggtgaactgcctgtgtgctcagcatgcccaaacctgcacgcgccctcgctgctttgcaaaggagggtttatgtgctaactggttttacaacccagcacttgcctttgaagggtttgatattccagactcttaccaagagggacacggtgtggtacctagttattaatagtaatcaattacggggtcattagttcatagcccatatatggagttccgcgttacataacttacggtaaatggcccgcctggctgaccgcccaacgacccccgcccattgacgtcaataatgacgtatgttcccatagtaacgccaatagggactttccattgacgtcaatgggtggagtatttacggtaaactgcccacttggcagtacatcaagtgtatcatatgccaagtacgccccctattgacgtcaatgacggtaaatggcccgcctggcattatgcccagtacatgaccttatgggactttcctacttggcagtacatctacgtattagtcatcgctattaccatggtgatgcggttttggcagtacatcaatgggcgtggatagcggtttgactcacggggatttccaagtctccaccccattgacgtcaatgggagtttgttttggcaccaaaatcaacgggactttccaaaatgtcgtaacaactccgccccattgacgcaaatgggcggtaggcgtgtacggtggcggatccgccgccaccatggccaccaccgccatgaggatgatcatcagcatcatcttcatcagcacctacgtgacccacatcaccctgtgccagaacatcaccgaggaattctaccagagcacctgtagcgccgtgtccaggggctacctgagcgccctgagaaccggctggtacaccagcgtggtgacaatcgagctgagcaagatccagaaaaacgtgtgcaacagcaccgacagcaaagtgaagctgatcaagcaagaactgggccgctacaacaacgccgtgattgaactgcagagcctgatgcagaacgagcccgccagcttcagcagggccaagaggggcatccccgagctgatccactaccccagaaacagcaccaagaggttctacggcctgatgggcaagaagaggaagcgcagattcctgggcttcctgctgggcatcggcagcgccatcgcttctggcgtggccgtgtctaaggtgctgcacctggaaggcgaagtgaacaagatcaagaacgccctgctgagcaccaacaaggctgtggtgtccctgagcaacggcgtgtccgtgctgaccagcaaggtgctggatctgaagaactacatcgacaaaaagctgctgcccaaggtcaacaaccacgactgcaggatcagcaacatcgagacagtgatcgagttccagcagaagaacaacaggctgctggaaatcgcccgcgagttcagcgtgaacgccggcatcaccacccccctgagcacctacatgctgaccaacagcgagctgctgagcctgatcaacgacatgcccatcaccaacgaccagaaaaagctgatgagcagcaacgtgcagatcgtgcgccagcagagctacagcatcatgagcgtggtgaaagaagaagtcattgcctacgtcgtgcagctgcccatctacggcgtgatcgacaccccctgctggaaggtgcacaccagccctctgtgcacaaccgacaacaaagagggcagcaacatctgcctgaccaggaccgacaggggctggtactgcgacaacgccggctccgtgtcattctttccacaagccgaaacatgcaaggtgcagagcaacagggtgttctgcgacaccatgaacagcctgaccctgcccaccgacgtgaacctgtgcaacaccgatatcttcaacaccaaatacgattgcaagatcatgacctccaagaccgacatcagcagcagcgtgatcaccagcatcggcgccatcgtgtcctgctacggcaagaccaagtgcaccgccagcaacaagaacaggggcatcatcaagaccttcagcaacggctgcgactacgtgtccaacaagggcgtggacaccgtgtccgtgggcaacaccctgtactacgtgaacaagctggaaggcaaggccctgtacatcaagggcgagcccatcatcaactactacgaccccctggtgttccccagcgacgagttcgacgcctctatcgctcaggtcaacgccaagatcaaccagagcctggccttcatcaggcgcagcgacgagctgctgcacagcgtggacgtgggcaagtccaccatcaacgtggtgatcacaaccatcatcatcgtgatcgtggtggtgatcctgatgctgatcgccgtgggcctgctgttctactgcaagacaaggtccacccccatcatgctgggcaaggaccagctgagcggcatcaacaacctgagcttctctaaataagtcgactatttcgagtacctctagggccgcttcgagcagacatgataagatacattgatgagtttggacaaaccacaactagaatgcagtgaaaaaaatgctttatttgtgaaatttgtgatgctattgctttatttgtaaccattataagctgcaataaacaagttaacaacaacaattgcattcattttatgtttcaggttcagggggagatgtgggaggttttttaaagcaagtaaaacctctacaaatgtggtaaaatcgaatctagatcctccttaagacaccctcagccttctaatgggactaaacaacaaaaatcaggcccatgtagcttgtcaaataaacttacctaatttttgctaagacgtctgggtcctgcgtttctatgtccaccaaagtcccctcttcccagctttggtacttccacttgtgcgcgcgagccagcttgcggatgtgcttgaaagataatgtggtctctcccaacagcttcccgttcaccagcaccagggccatgaagcggacacgaagagctctacctgcaaattatgaccctgtatatccatacgacgcccccgggtcttccacacaaccccctttttttaataacaagcaaggtctcactgagtcacccccaggaaccctggctgtcaatgtttcccctccactaaccttttctacgttaggtgccattaaactttccacaggtcccggactcaccctcaacgagggcaagttacaagccagcttagggcccggcctcatcacaaataccgagggccaaatcactgttggttt

SEQ ID NO: 28 - protein, 574 aa, Bovine respiratory syncytial virus
MATTAMRMIISIIFISTYVTHITLCQNITEEFYQSTCSAVSRGYLSALRTGWYTSVVTIELSKIQKNVCNSTDSKVKLIKQELGRYNNAVIELQSLMQNEPASFSRAKRGIPELIHYPRNSTKRFYGLMGKKRKRRFLGFLLGIGSAIASGVAVSKVLHLEGEVNKIKNALLSTNKAVVSLSNGVSVLTSKVLDLKNYIDKKLLPKVNNHDCRISNIETVIEFQQKNNRLLEIAREFSVNAGITTPLSTYMLTNSELLSLINDMPITNDQKKLMSSNVQIVRQQSYSIMSVVKEEVIAYVVQLPIYGVIDTPCWKVHTSPLCTTDNKEGSNICLTRTDRGWYCDNAGSVSFFPQAETCKVQSNRVFCDTMNSLTLPTDVNLCNTDIFNTKYDCKIMTSKTDISSSVITSIGAIVSCYGKTKCTASNKNRGIIKTFSNGCDYVSNKGVDTVSVGNTLYYVNKLEGKALYIKGEPIINYYDPLVFPSDEFDASIAQVNAKINQSLAFIRRSDELLHSVDVGKSTINVVITTIIIVIVVVILMLIAVGLLFYCKTRSTPIMLGKDQLSGINNLSFSK

SEQ ID NO: 29 - DNA, 600 bp, Equine herpesvirus 4
gcagactttggagcagcacaatttccggttgtggaccccatggaccttggtttggctggtaccgtggaaactaacgctccggaagttttggccagagcaaaatacaattcgaaggtagacatatggagcgccggaatagttctgtttgaaatgctcgcatatccatcaactctatttgaggacccgccgagtaccccacaagagtatgtaaaaagctgtcattctcaactactgagaataatatcaaagctaaagataaaccctgaggagtttccacgggaaccagagtctaggctcgtgcgcggatacatcgaatacgccagcctagagcgtaagccacatacgcgctatccttgcttccagcgcgtgaacctacacattgacggggaatttttgatccataaaatgctagcgttcaatgctgcgatgcgcccatccgcagaagagttgttgtcctacccaatgtttatgaatctgtaggatgactaacagatttggggtggagacggcgtgggcgatactgtataaagttgtactacttaccagcccagtcagtgtgctgtagtgccaccacctgtaaagctgtgataagctgcagtt

SEQ ID NO: 30 - DNA, 600 bp, Equine herpesvirus 4
agctgggggagtttgtactatagtgtattacatgcggcttgcaataactgcctggtttatgtttcgcaacattcaagcagacatgctaccgctaaacactttgcaacaattttttattgggtgtttggcctttggtagaactgtcgcgtttttggtggtagcatatactaccttatttatacgctccgagctgtttttcagcatgctagcacccaacgccgagcgagagtatataactcccatcattgcccacaagcttatgccacttattagcgtccgctctgccgtttgcttagtcataatatctaccgccgtttacgcagcagacgctatctgcgacacaattggatttgcgataccgcgcatgtggatgtgtattttaatgagatcaacctccatgaagcgtaactagggggcctcccactgaggcactaccggcttagcagctgactaacacagtataaaacgtgagaagaaatcagtctcatgcgccattagcgctaggctagttagcgtggaggaccggagcgctaccgccagcagtttcatccgcctggttacgggtttgttaacacctaccggtgttttaccgctaccata

SEQ ID NO: 31 - DNA, 442 bp, Equine herpesvirus 4
ggtacctctatttgaggacccgccgagtaccccacaagagtatgtaaaaagctgtcattctcaactactgagaataatatcaaagctaaagataaaccctgaggagtttccacgggaaccagagtctaggctcgtgcgcggatacatcgaatacgccagcctagagcgtaagccacatacgcgctatccttgcttccagcgcgtgaacctacacattgacggggaatttttgatccataaaatgctagcgttcaatgctgcgatgcgcccatccgcagaagagttgttgtcctacccaatgtttatgaatctgtaggatgactaacagatttggggtggagacggcgtgggcgatactgtataaagttgtactacttaccagcccagtcagtgtgctgtagtgccaccacctgtaaagctgtgataagctgcagttggatcc

SEQ ID NO: 32 - DNA, 467 bp, Equine herpesvirus 4
ggtaccactggtggtagcatatactaccttatttatacgctccgagctgtttttcagcatgctagcacccaacgccgagcgagagtatataactcccatcattgcccacaagcttatgccacttattagcgtccgctctgccgtttgcttagtcataatatctaccgccgtttacgcagcagacgctatctgcgacacaattggatttgcgataccgcgcatgtggatgtgtattttaatgagatcaacctccatgaagcgtaactagggggcctcccactgaggcactaccggcttagcagctgactaacacagtataaaacgtgagaagaaatcagtctcatgcgccattagcgctaggctagttagcgtggaggaccggagcgctaccgccagcagtttcatccgcctggttacgggtttgttaacacctaccggtgttttaccgctaccataggatcggatcc

SEQ ID NO: 33 - DNA, 37 bp, Artificial Sequence
  PRIMER
tttaaaggtacctctatttgaggacccgccgagtacc

SEQ ID NO: 34 - DNA, 42 bp, Artificial Sequence
  PRIMER
aaatttggatccaactgcagcttatcacagctttacaggtgg

SEQ ID NO: 35 - DNA, 47 bp, Artificial Sequence
  PRIMER
tttaaaggtaccactggtggtagcatatactacctttatttatacgc

SEQ ID NO: 36 - DNA, 38 bp, Artificial Sequence
  PRIMER
aaatttggatccgatcctatggtagcggtaaaacaccg

SEQ ID NO: 37 - DNA, 1776 bp, Artificial Sequence
  CPV VP2 Despliced ORF with BamHI and SalI Restriction Endonuclease Sites
ggatccgccgccaccatgtctgatggcgccgtgcagcctgatggcggacagcctgccgtccggaatgagagagccaccggcagcggcaatggatctggcggaggcggcggaggcggaagtggcggcgtcggcattagcaccggcaccttcaacaaccagaccgagttcaagttcctggaaaacggctgggtcgagatcaccgccaacagcagcagactcgtgcacctgaacatgcccgagagcgagaactaccggcgcgtcgtcgtgaacaacctggacaagaccgctgtcaacggcaacatggccctggacgatacccacgcccagattgtcacaccttggagcctcgtggatgccaatgcctggggggtgtggtttaaccccggcgactggcagctcattgtcaacaccatgagcgagctgcacctcgtctccttcgagcaggaaatcttcaacgtcgtgctgaaaactgtctccgagagcgccacacagccccccaccaaagtgtacaacaacgacctgaccgcctccctgatggtcgccctggacagcaacaacaccatgcccttcacccctgccgccatgcggagcgagacactgggcttctacccctggaagcccaccatccctaccccctggcggtactactttcaatgggacagaaccctgatccccagccacacaggcaccagcggcacccctaccaacatctaccacggcaccgaccccgacgacgtgcagttctacaccatcgagaacagcgtgcccgtgcatctgctgagaaccggcgacgaatttgccacaggcacattctttttcgactgcaaaccctgccggctgacccacacctggcagaccaatagagccctgggcctgcccccattcctgaactccctgcctcaggccgagggcggcaccaactttggctatatcggcgtgcagcaggacaagcggagaggagtcacacagatgggcaagaccaactacatcaccgaggccacaatcatgcggcctgccgaagtcggatacagcgccccctactacagcttcgaggccagcacccagggccccttcaagacacctattgccgccggaagaggcggagcccagaccgatgagaatcagggcgccgacggcaaccccagatacgcctttggcagacagcacggccagaaaaccaccaccaccggcgagacacccgaacgcttcacctatatcgcccaccaggacaccggcagataccccgagggcgactggattcagaacatcaacttcaacctgcctgtcaccgacgacaacgtgctgctgcccacagatcccatcggcggcaagaccggcatcaactacaccaatatcttcaacacctacggccctctgaccgccctgaacaacgtgccccccgtgtaccccaacggacagatctgggacaaggaattcgacaccgacctgaagccccggctgcacgtcaacgcccctttcgtctgccagaacaactgccctggccaactcttcgtcaaagtggcccccaacctgaccaatgaatatgaccctgacgccagcgccaacatgagccggattgtcacctacagcgacttttggtggaagggaaaactcgtgttcaaggccaagctgcgggcctctcacacctggaaccccatccagcaaatgagcatcaacgtggacaaccagttcaactacgtgcccagcaacatcggcggaatggaaattgtcttcgaacgctcccagctggcccccagaaagctgtactaagtcgac

SEQ ID NO: 38 - DNA, 1776 bp, Artificial Sequence
  CPV VP2 Gen0.95 ORF with BamHI and SalI Restriction Endonuclease Sites
ggatccgccgccaccatgtctgatggcgccgtgcagcctgatggcggacagcctgctgtgcggaatgagagagccaccggcagcggcaatggatctggcggaggcggcggagggggaagtggcggagtgggaattagcaccggcaccttcaacaaccagaccgagttcaagttcctggaaaacggctgggtggaaatcaccgccaacagcagcagactggtgcacctgaacatgcccgagagcgagaactaccggcgggtggtcgtgaacaacctggacaagaccgccgtgaacggcaacatggccctggacgatacccacgcccagatcgtgacaccctggtccctggtggatgccaatgcctggggcgtgtggttcaaccccggcgactggcagctgatcgtgaacaccatgagcgagctgcacctggtgtccttcgagcaggaaatcttcaacgtggtgctgaaaaccgtgtccgagagcgccacacagccccccaccaaggtgtacaacaacgacctgaccgcctccctgatggtggctctggacagcaacaacaccatgcccttcacccctgccgccatgcggagcgagacactgggcttctacccctggaagcccaccatccctaccccctggcggtactacttccagtgggacagaaccctgatccccagccacacaggcaccagcggcacccctaccaacatctaccacggcaccgaccccgacgacgtgcagttctacaccatcgagaacagcgtgcccgtgcatctgctgagaaccggcgacgagttcgctaccggaacattcttcttcgactgcaaaccctgccggctgacccacacctggcagaccaatagagccctgggcctgccccccttcctgaactctctgcctcaggctgagggcggcaccaacttcggctacatcggcgtgcagcaggacaagcggagaggcgtgacccagatgggcaaaaccaactacatcaccgaggccacaatcatgcggcctgccgaagtgggctacagcgccccctactacagcttcgaggccagcacccagggccccttcaagacacctattgccgccggaagaggcggagcccagaccgatgagaatcagggagctgacggcaaccccagatacgcctttggcagacagcacggccagaaaaccaccaccaccggcgagacacccgagcggttcacctacattgcccaccaggacaccggcagataccccgagggcgattggattcagaacatcaacttcaacctgcccgtgaccgacgacaacgtgctgctgcccacagatcccatcggcggcaagaccggcatcaactacaccaatatcttcaacacctacggccctctgaccgccctgaacaacgtgcccccagtgtaccccaacggccagatttgggacaaagagttcgacaccgacctgaagccccggctgcatgtgaacgcccctttcgtgtgccagaacaactgccctggccagctgtttgtgaaggtggcccccaacctgaccaacgagtacgaccctgacgccagcgccaacatgagccggatcgtgacctacagcgacttctggtggaagggcaagctggtgttcaaggccaagctgcgggcctctcacacctggaaccccatccagcagatgagcatcaacgtggacaaccagttcaactacgtgcccagcaacatcggcggaatggaaatcgtgtttgagagatcccagctggcccccagaaagctgtactgagtcgac

SEQ ID NO: 39 - DNA, 1776 bp, Artificial Sequence; identical to SEQ ID NO: 37
  NUCLEOTIDE SEQUENCE OF TRANSFER PLASMID EHV-4 p430 CPV VP2 (Despliced  )EXPRESSION CASSETTE

SEQ ID NO: 40 - DNA, 1776 bp, Artificial Sequence; identical to SEQ ID NO: 38
  NUCLEOTIDE SEQUENCE OF TRANSFER PLASMID EHV-4 p430 CPV VP2 (Gen 0.95) EXPRESSION CASSETTE

SEQ ID NO: 41 - DNA, 2502 bp, Artificial Sequence
  NUCLEOTIDE SEQUENCE OF TRANSFER PLASMID EHV-4 pp455 CPV VP2 (Gen0.95) EXPRESSION CASSETTE
actggtggtagcatatactaccttatttatacgctccgagctgtttttcagcatgctagcacccaacgccgagcgagagtatataactcccatcattgcccacaagcttatgccacttattagcgtccgctctgccgtttgcttagtcataatatctaccgccgtttacgcagcagacgctatctgcgacacaattggatttgcgataccgcgcatgtggatgtgtattttaatgagatcaacctccatgaagcgtaactagggggcctcccactgaggcactaccggcttagcagctgactaacacagtataaaacgtgagaagaaatcagtctcatgcgccattagcgctaggctagttagcgtggaggaccggagcgctaccgccagcagtttcatccgcctggttacgggtttgttaacacctaccggtgttttaccgctaccataggatcggatccgccgccaccatgtctgatggcgccgtgcagcctgatggcggacagcctgctgtgcggaatgagagagccaccggcagcggcaatggatctggcggaggcggcggagggggaagtggcggagtgggaattagcaccggcaccttcaacaaccagaccgagttcaagttcctggaaaacggctgggtggaaatcaccgccaacagcagcagactggtgcacctgaacatgcccgagagcgagaactaccggcgggtggtcgtgaacaacctggacaagaccgccgtgaacggcaacatggccctggacgatacccacgcccagatcgtgacaccctggtccctggtggatgccaatgcctggggcgtgtggttcaaccccggcgactggcagctgatcgtgaacaccatgagcgagctgcacctggtgtccttcgagcaggaaatcttcaacgtggtgctgaaaaccgtgtccgagagcgccacacagccccccaccaaggtgtacaacaacgacctgaccgcctccctgatggtggctctggacagcaacaacaccatgcccttcacccctgccgccatgcggagcgagacactgggcttctacccctggaagcccaccatccctaccccctggcggtactacttccagtgggacagaaccctgatccccagccacacaggcaccagcggcacccctaccaacatctaccacggcaccgaccccgacgacgtgcagttctacaccatcgagaacagcgtgcccgtgcatctgctgagaaccggcgacgagttcgctaccggaacattcttcttcgactgcaaaccctgccggctgacccacacctggcagaccaatagagccctgggcctgccccccttcctgaactctctgcctcaggctgagggcggcaccaacttcggctacatcggcgtgcagcaggacaagcggagaggcgtgacccagatgggcaaaaccaactacatcaccgaggccacaatcatgcggcctgccgaagtgggctacagcgccccctactacagcttcgaggccagcacccagggccccttcaagacacctattgccgccggaagaggcggagcccagaccgatgagaatcagggagctgacggcaaccccagatacgcctttggcagacagcacggccagaaaaccaccaccaccggcgagacacccgagcggttcacctacattgcccaccaggacaccggcagataccccgagggcgattggattcagaacatcaacttcaacctgcccgtgaccgacgacaacgtgctgctgcccacagatcccatcggcggcaagaccggcatcaactacaccaatatcttcaacacctacggccctctgaccgccctgaacaacgtgcccccagtgtaccccaacggccagatttgggacaaagagttcgacaccgacctgaagccccggctgcatgtgaacgcccctttcgtgtgccagaacaactgccctggccagctgtttgtgaaggtggcccccaacctgaccaacgagtacgaccctgacgccagcgccaacatgagccggatcgtgacctacagcgacttctggtggaagggcaagctggtgttcaaggccaagctgcgggcctctcacacctggaaccccatccagcagatgagcatcaacgtggacaaccagttcaactacgtgcccagcaacatcggcggaatggaaatcgtgtttgagagatcccagctggcccccagaaagctgtactgagtcgactatttcgagtacctctagggccgcttcgagcagacatgataagatacattgatgagtttggacaaaccacaactagaatgcagtgaaaaaaatgctttatttgtgaaatttgtgatgctattgctttatttgtaaccattataagctgcaataaacaagttaacaacaacaattgcattcattttatgtttcaggttcagggggagatgtgggaggttttttaaagcaagtaaaacctctacaaatgtggtaaaatcgaatctagatcctc

SEQ ID NO: 42 - DNA, 2304 bp, Artificial Sequence
  NUCLEOTIDE SEQUENCE OF TRANSFER PLASMID EHV-4 p430 RabG (n) EXPRESSION CASSETTE
ctctatttgaggacccgccgagtaccccacaagagtatgtaaaaagctgtcattctcaactactgagaataatatcaaagctaaagataaaccctgaggagtttccacgggaaccagagtctaggctcgtgcgcggatacatcgaatacgccagcctagagcgtaagccacatacgcgctatccttgcttccagcgcgtgaacctacacattgacggggaatttttgatccataaaatgctagcgttcaatgctgcgatgcgcccatccgcagaagagttgttgtcctacccaatgtttatgaatctgtaggatgactaacagatttggggtggagacggcgtgggcgatactgtataaagttgtactacttaccagcccagtcagtgtgctgtagtgccaccacctgtaaagctgtgataagctgcagttggatccgccgccaccatggtaccggttcctcaggctctcctgtttgtaccccttctggtttttccattgtgttttgggaaattccctatttacacgataccagacaagcttggtccctggagcccgattgacatacatcacctcagctgcccaaacaatttggtagtggaggacgaaggatgcaccaacctgtcagggttctcctacatggaacttaaagttggatacatctcagccataaaaatgaacgggttcacttgcacaggcgttgtgacggaggctgaaacctacactaacttcgttggttatgtcacaaccacgttcaaaagaaagcatttccgcccaacaccagatgcatgtagagccgcgtacaactggaagatggccggtgaccccagatatgaagagtctctacacaatccgtaccctgactaccactggcttcgaactgtaaaaaccaccaaggagtctctcgttatcatatctccaagtgtggcagatttggacccatatgacagatcccttcactcgagggtcttccctggcgggaagtgctcaggagtagcggtgtcttctacctactgctccactaaccacgattacaccatttggatgcccgagaatccgagactagggatgtcttgtgacatttttaccaatagtagagggaagagagcatccaaagggagtgagacttgcggctttgtagatgaaagaggcctatataagtctttaaaaggagcatgcaaactcaagttatgtggagttctcggacttagacttatggatggaacatgggtctcgatgcaaacatcaaatgaaaccaaatggtgccctcccggtcagttgatcaatttgcacgactttcgctcagacgaaattgagcaccttgttgtagaggagttggtcaagaagagagaggagtgtctggatgcactagagtccatcatgaccaccaagtcagtaagtttcagacgtctcagtcatttaagaaaacttgtccctgggtttggaaaagcatataccatattcaacaagaccttgatggaagccgatgctcactacaagtcagtcagaacttggaatgagatcatcccttcaaaagggtgtttaagagttggggggaggtgtcatcctcatgtaaacggggtatttttcaatggtataatattaggacctgacggcaatgtcttaatcccagagatgcaatcatccctcctccagcaacatatggagttgttggtatcctcggttatcccccttatgcaccccctggcagacccgtctaccgttttcaagaacggtgacgaggctgaggattttgttgaagttcaccttcccgatgtgcacgaacggatctcaggagttgacttgggtctcccgaactgggggaagtatgtattactgagtgcaggggccctgactgccttgatgttgataattttcctgatgacatgctggagaagagtcaatcgatcggaacctacacaacacaatctcagagggacagggagggaggtgtcagtcactccccaaagcgggaagatcatatcttcatgggaatcatacaagagcgggggtgagaccggactgtgagtcgactatttcgagtacctctagggccgcttcgagcagacatgataagatacattgatgagtttggacaaaccacaactagaatgcagtgaaaaaaatgctttatttgtgaaatttgtgatgctattgctttatttgtaaccattataagctgcaataaacaagttaacaacaacaattgcattcattttatgtttcaggttcagggggagatgtgggaggttttttaaagcaagtaaaacctctacaaatgtggtaaaatcgaatctagatcctc

SEQ ID NO: 43 - DNA, 2328 bp, Artificial Sequence
  NUCLEOTIDE SEQUENCE OF TRANSFER PLASMID EHV-4 p455 RabG (n)       EXPRESSION CASSETTE
actggtggtagcatatactaccttatttatacgctccgagctgtttttcagcatgctagcacccaacgccgagcgagagtatataactcccatcattgcccacaagcttatgccacttattagcgtccgctctgccgtttgcttagtcataatatctaccgccgtttacgcagcagacgctatctgcgacacaattggatttgcgataccgcgcatgtggatgtgtattttaatgagatcaacctccatgaagcgtaactagggggcctcccactgaggcactaccggcttagcagctgactaacacagtataaaacgtgagaagaaatcagtctcatgcgccattagcgctaggctagttagcgtggaggaccggagcgctaccgccagcagtttcatccgcctggttacgggtttgttaacacctaccggtgttttaccgctaccataggatcggatccgccgccaccatggtaccggttcctcaggctctcctgtttgtaccccttctggtttttccattgtgttttgggaaattccctatttacacgataccagacaagcttggtccctggagcccgattgacatacatcacctcagctgcccaaacaatttggtagtggaggacgaaggatgcaccaacctgtcagggttctcctacatggaacttaaagttggatacatctcagccataaaaatgaacgggttcacttgcacaggcgttgtgacggaggctgaaacctacactaacttcgttggttatgtcacaaccacgttcaaaagaaagcatttccgcccaacaccagatgcatgtagagccgcgtacaactggaagatggccggtgaccccagatatgaagagtctctacacaatccgtaccctgactaccactggcttcgaactgtaaaaaccaccaaggagtctctcgttatcatatctccaagtgtggcagatttggacccatatgacagatcccttcactcgagggtcttccctggcgggaagtgctcaggagtagcggtgtcttctacctactgctccactaaccacgattacaccatttggatgcccgagaatccgagactagggatgtcttgtgacatttttaccaatagtagagggaagagagcatccaaagggagtgagacttgcggctttgtagatgaaagaggcctatataagtctttaaaaggagcatgcaaactcaagttatgtggagttctcggacttagacttatggatggaacatgggtctcgatgcaaacatcaaatgaaaccaaatggtgccctcccggtcagttgatcaatttgcacgactttcgctcagacgaaattgagcaccttgttgtagaggagttggtcaagaagagagaggagtgtctggatgcactagagtccatcatgaccaccaagtcagtaagtttcagacgtctcagtcatttaagaaaacttgtccctgggtttggaaaagcatataccatattcaacaagaccttgatggaagccgatgctcactacaagtcagtcagaacttggaatgagatcatcccttcaaaagggtgtttaagagttggggggaggtgtcatcctcatgtaaacggggtatttttcaatggtataatattaggacctgacggcaatgtcttaatcccagagatgcaatcatccctcctccagcaacatatggagttgttggtatcctcggttatcccccttatgcaccccctggcagacccgtctaccgttttcaagaacggtgacgaggctgaggattttgttgaagttcaccttcccgatgtgcacgaacggatctcaggagttgacttgggtctcccgaactgggggaagtatgtattactgagtgcaggggccctgactgccttgatgttgataattttcctgatgacatgctggagaagagtcaatcgatcggaacctacacaacacaatctcagagggacagggagggaggtgtcagtcactccccaaagcgggaagatcatatcttcatgggaatcatacaagagcgggggtgagaccggactgtgagtcgactatttcgagtacctctagggccgcttcgagcagacatgataagatacattgatgagtttggacaaaccacaactagaatgcagtgaaaaaaatgctttatttgtgaaatttgtgatgctattgctttatttgtaaccattataagctgcaataaacaagttaacaacaacaattgcattcattttatgtttcaggttcagggggagatgtgggaggttttttaaagcaagtaaaacctctacaaatgtggtaaaatcgaatctagatcctc

SEQ ID NO: 44 - DNA, 24 bp, Artificial Sequence
  PRIMER
ctggttttacaacccagcacttgc

SEQ ID NO: 45 - DNA, 22 bp, Artificial Sequence
  PRIMER
gactcctctccgcttgtcctgc

SEQ ID NO: 46 - DNA, 24 bp, Artificial Sequence
  PRIMER
ctggttttacaacccagcacttgc

SEQ ID NO: 47 - DNA, 22 bp, Artificial Sequence
  PRIMER
cgatgtagccgaagttggtgcc